European Patent Application EP 4 170 025 A1, published April 26, 2023. Title: NOVEL URIDINE DIPHOSPHATE GLYCOSYLTRANSFERASE AND USE THEREOF. Applicant: CJ CheilJedang Corporation. The sequence listing filed with the application follows.

SEQUENCE LISTING (6 sequences)

SEQ ID NO: 1 - protein, 463 aa, Unknown
  UGT-B
MDGDGNSSSSSSPLHVVICPWLALGHLLPCLDIAERLASRGHRVSFVSTPRNIARLPPLRPAVAPLVEFVALPLPHVDGLPEGAESTNDVPYDKFELHRKAFDGLAAPFSEFLRAACAEGAGSRPDWLIVDTFHHWAAAAAVENKVPCVMLLLGAATVIAGFARGVSEHAAAAVGKERPAAEAPSFETERRKLMTTQNASGMTVAERYFLTLMRSDLVAIRSCAEWEPESVAALTTLAGKPVVPLGLLPPSPEGGRGVSKEDATVRWLDAQPTKSVVYVALGSEVPLGAKEVHELALGLELAGTRFLWSLRKPSGVSDADILPSGFEERTRGRGLVTMGWVPQISVLAHGAVGAFLTHCGWNSIIEGLQFGHPLVMLPIFGDQGPNARMMEGRKVGVQVPRDESNGSFDREGVATTVRAVAVEEEGNRIFTANAKKMQEIVADKGCHDKYVDKFIQKLRSYME

SEQ ID NO: 2 - protein, 458 aa, Unknown
  UGT-A
MENKTETTVRRRRRIILFPVPFQGHINPILQLANVLYSKGFSITIFHTNFNKPKTSNYPHFTFRFILDNDPQDERISNLPTHGPLAGMRIPIINEHGADELRRELELLMLASEEDEEVSCLITDALWYFAQSVADSLNLRRLVLMTSSLFNFHAHVSLPQFDELGYLDPDDKTRLEEQASGFPMLKVKDIKSAYSNWQILKEILGKMIKQTKASSGVIWNSFKELEESELETVIREIPAPSFLIPLPKHLTASSSSLLDHDRTVFQWLDQQPPSSVLYVSFGSTSEVDEKDFLEIARGLVDSKQSFLWVVRPGFVKGSTWVEPLPDGFLGERGRIVKWVPQQEVLAHGAIGAFWTHSGWNSTLESVCEGVPMIFSDFGLDQPLNARYMSDVLKVGVYLENGWERGEIANAIRRVMVDEEGEYIRQNARVLKQKADVSLMKGGSSYESLESLVSYISSL

SEQ ID NO: 3 - protein, 808 aa, Unknown
  Sucrose synthase
MAAKLARLHSLRERLGATFSSHPNELIALFSRYVNQGKGMLQRHQLLAEFDALIEADKEKYAPFEDILRAAQEAIVLPPWVALAIRPRPGVWDYIRVNVSELAVEELSVSEYLAFKEQLVDGHTNSNFVLELDFEPFNASFPRPSMSKSIGNGVQFLNRHLSSKLFQDKESLYPLLNFLKAHNHKGTTMMLNDRIQSLRGLQSSLRKAEEYLMGIPQDTPYSEFNHRFQELGLEKGWGDCAKRVLDTIHLLLDLLEAPDPANLEKFLGTIPMMFNVVILSPHGYFAQSNVLGYPDTGGQVVYILDQVRALENEMLLRIKQQGLDITPKILIVTRLLPDAVGTTCGQRVEKVIGTEHTDILRVPFRSENGILRKWISRFDVWPFLETYTEDVANEIMREMQAKPDLIIGNYSDGNLVATLLAHKLGVTQCTIAHALEKTKYPNSDIYLDKFDSQYHFSCQFTADLIAMNHTDFIITSTFQEIAGSKDTVGQYESHIAFTLPGLYRVVHGIDVFDPKFNIVSPGADMSVYFPYTEADKRLTAFHPEIEELLYSEVENDEHKFVLKDKNKPIIFSMARLDRVKNMTGLVEMYGKNAHLRDLANLVIVCGDHGNQSKDREEQAEFKKMYGLIDQYKLKGHIRWISAQMNRVRNGELYRYICDTKGVFVQPAFYEAFGLTVIEAMTCGLPTIATCHGGPAEIIVDGVSGLHIDPYHSDKAADILVNFFEKCKQDSTYWDNISQGGLQRIYEKYTWKLYSERLMTLTGVYGFWKYVSNLERRETRRYIEMFYALKYRSLASAVPLAVDGESTSK

SEQ ID NO: 4 - DNA, 1392 bp, Unknown
  UGT-B
atggatggtgacggcaactcctccagttcgagtagtccgctgcatgtagttatatgcccgtggttagccttgggccatttactgccgtgtctggatattgccgaacgcctggcgagccgcggccaccgtgtctcatttgtctccacgccgcgcaacatcgcgcgcttgccgccgctgcgccccgctgtggcgccgctcgtcgaatttgtcgccctgcctctaccgcatgtcgatggtttgcctgaaggcgcagaaagtacaaacgatgtcccatacgacaaattcgagttacatcgcaaagcctttgatggcctcgctgcacccttttcagagtttctgcgtgcagcttgtgccgagggcgctggatctcggcccgattggcttatagtggatacctttcaccactgggcagccgcggctgccgtcgaaaataaagttccgtgcgttatgcttttgctgggagctgcgacagtgatcgcaggtttcgctcgaggtgtgtctgagcacgccgctgcagccgtcgggaaagagcgaccggcagcggaagcgccatcttttgagactgaaaggaggaagctgatgaccacgcagaatgcaagcgggatgacggtagccgaacgctacttcttaacgttaatgcgtagcgatctcgtggccattcggagctgtgctgagtgggagccagagagcgtcgccgcgttaaccaccttagcgggcaagccagtcgtccctttgggtttgctaccaccgtcgcccgaaggaggtcgcggtgtgagcaaggaggatgcaaccgtgcgttggctcgatgcccagccgaccaaatcagtggtttatgtcgcgctaggctcggaagtcccactgggagccaaggaagtacatgaacttgccttaggccttgagttagcagggacacgcttcctttggtctctgcgcaaaccttctggcgtaagtgatgcagacatcctcccttcgggttttgaagagcggacccgcggccgtggtcttgtgacgatgggctgggttcctcagattagcgtactggcacacggtgcagtaggtgcattcctgactcattgtggatggaactctatcatagaggggttacaatttgggcatcctttagtgatgttgcctatctttggtgaccaaggtcccaatgcgcgtatgatggaggggagaaaagttggagtgcaggtgccaagagatgaatccaatggaagtttcgacagagaaggcgtcgctacaaccgttcgggcggtcgctgtcgaggaagaaggtaatagaattttcactgctaatgccaaaaaaatgcaagagatcgttgcggacaaaggatgccatgacaagtatgtcgataaatttattcagaaactgagatcttatatggagtga

SEQ ID NO: 5 - DNA, 1377 bp, Unknown
  UGT-A
atggaaaataaaacggagaccaccgttcgccggcgccggagaataatattattcccggtaccatttcaaggccacattaacccaattcttcagctagccaatgtgttgtactctaaaggattcagtatcaccatctttcacaccaacttcaacaaacccaaaacatctaattaccctcacttcactttcagattcatcctcgacaacgacccacaagacgaacgcatttccaatctaccgactcatggtccgctcgctggtatgcggattccgattatcaacgaacacggagctgacgaattacgacgcgaactggaactgttgatgttagcttctgaagaagatgaagaggtatcgtgtttaatcacggatgctctttggtacttcgcgcaatctgttgctgacagtcttaacctccgacggcttgttttgatgacaagcagcttgtttaattttcatgcacatgtttcacttcctcagtttgatgagcttggttacctcgatcctgatgacaaaacccgtttggaagaacaagcgagtgggtttcctatgctaaaagtgaaagacatcaagtctgcgtattcgaactggcaaatactcaaagagatattagggaagatgataaaacaaacaaaagcatcttcaggagtcatctggaactcatttaaggaactcgaagagtctgagctcgaaactgttatccgtgagatcccggctccaagtttcttgataccactccccaagcatttgacagcctcttccagcagcttactagaccacgatcgaaccgtttttcaatggttagaccaacaaccgccaagttcggtactgtatgttagttttggtagtactagtgaagtggatgagaaagatttcttggaaatagctcgtgggttggttgatagcaagcagtcgtttttatgggtggttcgacctgggtttgtcaagggttcgacgtgggtcgaaccgttgccagatgggttcttgggtgaaagaggacgtattgtgaaatgggttccacagcaagaagtgctagctcatggagcaataggcgcattctggactcatagcggatggaactctacgttggaaagcgtttgtgaaggtgttcctatgattttctcggattttgggctcgatcaaccgttgaatgctagatacatgagtgatgttttgaaggtaggggtgtatttggaaaatgggtgggaaagaggagagatagcaaatgcaataagaagagttatggtggatgaagaaggagaatacattagacagaatgcaagagttttgaaacaaaaggcagatgtttctttgatgaagggtggttcgtcttacgaatcattagagtctctagtttcttacatttcatcgttgtaa

SEQ ID NO: 6 - DNA, 2427 bp, Unknown
  Sucrose synthase
atggctgccaagctagctcgcctccacagtctccgcgaacgcctcggtgccaccttctcgtctcatcccaatgagttgattgcactcttctctaggtatgttaaccagggaaagggaatgctccagcgtcaccagctgcttgcggagttcgatgccttgatcgaagctgacaaagagaaatatgctccctttgaagacattctccgggctgctcaggaagccattgtgctgccgccctgggttgcactggccatcaggccaaggcctggtgtctgggactacattcgggtgaatgtaagtgagttggcagtggaagagctgagtgtttctgagtacttggcattcaaggaacagcttgttgatggacacaccaacagcaactttgttcttgagcttgattttgagcccttcaatgcctccttcccgcgcccgtccatgtccaagtccatcggaaatggggtgcagttccttaaccgtcacctgtcgtccaagttgttccaggacaaggagagcctctaccccttgctgaacttcctgaaagcccataaccacaagggcacgacaatgatgctgaatgacagaattcagagccttcgtgggctccaatcatcccttagaaaggcagaagaatatctgatgggcattcctcaagacacgccctactcggagttcaaccacaggttccaagagctcggtttggagaagggttggggtgactgtgcaaagcgtgtgcttgacaccatccacttgcttcttgaccttcttgaggcccctgatccggccaacttggagaagttccttggaactattccaatgatgttcaatgttgttatcctgtctccgcatggatactttgcccaatccaatgtgttgggataccctgatactggtggtcaggttgtgtacattttggaccaagtccgcgctttggagaatgagatgcttttgaggatcaagcagcaaggccttgatatcacacctaagatcctcattgtaaccaggctgttgcctgatgctgttggtactacatgcggccagcgtgtggagaaggttattggaactgagcacactgacattcttcgtgttccattcaggagtgagaatggtatcctccgcaagtggatctcccgttttgatgtctggccattcctggaaacatacactgaggatgttgcaaacgaaattatgagggaaatgcaagccaaacctgatctcatcattggcaattacagtgatggaaaccttgttgccactctgctggctcacaaattaggagttacccagtgtaccattgctcatgccttggagaaaaccaaataccccaactcagacatatacttggacaagtttgacagccagtaccacttctcatgccaattcactgctgatcttatcgccatgaatcacactgatttcatcatcaccagtacattccaagaaattgctggaagcaaggacactgtggggcagtatgaatcacacattgcattcacccttcctgggctttaccgagttgtgcatggcatagatgtttttgatcccaagttcaacattgtctctcctggagctgacatgagtgtctacttcccgtacaccgaggctgacaagaggctcactgctttccaccctgaaattgaggagcttctctacagtgaagtcgagaacgatgaacacaagtttgtattgaaggacaagaacaagccaatcatcttctccatggctcgtcttgaccgagtgaagaacatgacaggtctggttgagatgtatggtaagaatgcacatctcagggatttggcaaaccttgtgattgtttgtggtgaccacggcaatcagtccaaggacagggaggagcaggctgagttcaagaagatgtacggtctcattgaccagtacaagttgaaggggcatatccgctggatctcagctcagatgaaccgtgttcgtaacggggagttgtaccgatacatttgtgacaccaagggagtctttgtccagcctgcattctatgaagcgtttggtctgactgtcatcgaagccatgacatgtggtttgccaacaatcgcaacatgccatggtggccctgctgagattattgttgatggggtgtctggtctgcacattgatccttaccacagtgacaaggctgctgatatcttggtcaacttctttgagaagtgcaagcaggattcaacctactgggacaatatttcacagggaggtctgcagaggatttacgagaagtacacctggaagctgtactctgagaggctgatgaccttgactggtgtatacggattctggaagtacgtaagcaaccttgagaggcgcgagactcgccgttacattgagatgttctatgctctgaaataccgcagcctggccagcgccgtcccattggctgtcgatggagagagcacatccaagtaa